European Patent Application EP 4 585 615 A1, published July 16, 2025. Title: MULTISPECIFIC ANTIBODY BINDING TO BCMA, GPRC5D AND CD3, AND USE THEREOF. Applicant: BEIJING MABWORKS BIOTECH CO., LTD. Application EP EP22957767.1, filed September 9, 2022. The sequence listing filed with the application follows.

SEQUENCE LISTING (37 sequences)

SEQ ID NO: 1 - protein, 5 aa, synthetic construct
NHIIH

SEQ ID NO: 2 - protein, 17 aa, synthetic construct
YINPYPGYHGYNDKFSG

SEQ ID NO: 3 - protein, 12 aa, synthetic construct
DGYYRDQDVLDY

SEQ ID NO: 4 - protein, 11 aa, synthetic construct
KASQDISQYLN

SEQ ID NO: 5 - protein, 7 aa, synthetic construct
YTSGLHP

SEQ ID NO: 6 - protein, 9 aa, synthetic construct
QQGYALPWT

SEQ ID NO: 7 - protein, 121 aa, synthetic construct
QVQLVQSGAEVKKPGASVKVSCKASGYTFTNHIIHWVRQAPGQGLEWMGYINPYPGYHGYNDKFSGRATMTSDTSTSTVYMELSSLRSEDTAVYYCARDGYYRDQDVLDYWGQGTLVTVSS

SEQ ID NO: 8 - protein, 107 aa, synthetic construct
DIQMTQSPSSLSASVGDRVTITCKASQDISQYLNWYQQKPGKAPKLLIYYTSGLHPGVPSRFSGSGSGTDFTFTISSLEPEDEATYYCQQGYALPWTFGQGTKLTAK

SEQ ID NO: 9 - protein, 5 aa, synthetic construct
DFAMH

SEQ ID NO: 10 - protein, 17 aa, synthetic construct
GITWNSGSVGYADSVKG

SEQ ID NO: 11 - protein, 14 aa, synthetic construct
DRSGYGHYYYGMDV

SEQ ID NO: 12 - protein, 11 aa, synthetic construct
RASTSVSHNVA

SEQ ID NO: 13 - protein, 7 aa, synthetic construct
GASTKVT

SEQ ID NO: 14 - protein, 9 aa, synthetic construct
QHYINWPLT

SEQ ID NO: 15 - protein, 123 aa, synthetic construct
EVQLVESGGGLVQPGRSLRLSCAASGFTFDDFAMHWVRQAPGKGLEWVSGITWNSGSVGYADSVKGRFTISRDNAKKSLYLQMNSLRAEDTALYYCAKDRSGYGHYYYGMDVWGQGTTVTVAS

SEQ ID NO: 16 - protein, 107 aa, synthetic construct
EIVMTQSPATLSVSPGERATLSCRASTSVSHNVAWYQQKPGQAPRLLIYGASTKVTGIPARFSGSGSGTEFTLTISSLQSEDFAVYYCQHYINWPLTFGGGTKVEIK

SEQ ID NO: 17 - protein, 6 aa, synthetic construct
SDYAWN

SEQ ID NO: 18 - protein, 16 aa, synthetic construct
YISYSGSATYSPSLKS

SEQ ID NO: 19 - protein, 14 aa, synthetic construct
GGIAGRGRWGAMDY

SEQ ID NO: 20 - protein, 11 aa, synthetic construct
KASQNVGTNVA

SEQ ID NO: 21 - protein, 7 aa, synthetic construct
SASYRDS

SEQ ID NO: 22 - protein, 9 aa, synthetic construct
QQYKSYPLT

SEQ ID NO: 23 - protein, 123 aa, synthetic construct
QVQLQESGPGLVKPSETLSLTCTVSGYSITSDYAWNWIRQPPGKGLEWMGYISYSGSATYSPSLKSRITISRDTSKNQFSLKLSSVTAADTAVYYCARGGIAGRGRWGAMDYWGQGTTVTVSS

SEQ ID NO: 24 - protein, 107 aa, synthetic construct
DIQMTQSPSSLSASVGDRVTITCKASQNVGTNVAWYQQKPGQSPKALIYSASYRDSGVPDRFSGSGSGTDFTLTISSLQPEDFATYYCQQYKSYPLTFGQGTRLEIK

SEQ ID NO: 25 - protein, 330 aa, synthetic construct
  VARIANT 249: note = W or S
  VARIANT 251: note = L or A
  VARIANT 290: note = Y or V
ASTKGPSVFPLAPSSKSTSGGTAALGCLVKDYFPEPVTVSWNSGALTSGVHTFPAVLQSSGLYSLSSVVTVPSSSLGTQTYICNVNHKPSNTKVDKKVEPKSCDKTHTCPPCPAPEAAGGPSVFLFPPKPKDTLMISRTPEVTCVVVDVSHEDPEVKFNWYVDGVEVHNAKTKPREEQYASTYRVVSVLTVLHQDWLNGKEYKCKVSNKALPAPIEKTISKAKGQPREPQVYTLPPSREEMTKNQVSLXCXVKGFYPSDIAVEWESNGQPENNYKTTPPVLDSDGSFFLXSKLTVDKSRWQQGNVFSCSVMHEALHNHYTQKSLSLSPGK

SEQ ID NO: 26 - protein, 107 aa, synthetic construct [sequence omitted]

SEQ ID NO: 27 - protein, 716 aa, synthetic construct
QVQLVQSGAEVKKPGASVKVSCKASGYTFTNHIIHWVRQAPGQGLEWMGYINPYPGYHGYNDKFSGRATMTSDTSTSTVYMELSSLRSEDTAVYYCARDGYYRDQDVLDYWGQGTLVTVSSGGGGSGGGGSGGGGSGGGGSDIQMTQSPSSLSASVGDRVTITCKASQDISQYLNWYQQKPGKAPKLLIYYTSGLHPGVPSRFSGSGSGTDFTFTISSLEPEDEATYYCQQGYALPWTFGQGTKLTAKGGGGSGGGGSGGGGSEVQLVESGGGLVQPGRSLRLSCAASGFTFDDFAMHWVRQAPGKGLEWVSGITWNSGSVGYADSVKGRFTISRDNAKKSLYLQMNSLRAEDTALYYCAKDRSGYGHYYYGMDVWGQGTTVTVASASTKGPSVFPLAPSSKSTSGGTAALGCLVKDYFPEPVTVSWNSGALTSGVHTFPAVLQSSGLYSLSSVVTVPSSSLGTQTYICNVNHKPSNTKVDKKVEPKSCDKTHTCPPCPAPEAAGGPSVFLFPPKPKDTLMISRTPEVTCVVVDVSHEDPEVKFNWYVDGVEVHNAKTKPREEQYASTYRVVSVLTVLHQDWLNGKEYKCKVSNKALPAPIEKTISKAKGQPREPQVYTLPPSREEMTKNQVSLWCLVKGFYPSDIAVEWESNGQPENNYKTTPPVLDSDGSFFLYSKLTVDKSRWQQGNVFSCSVMHEALHNHYTQKSLSLSPGK

SEQ ID NO: 28 - protein, 214 aa, synthetic construct
EIVMTQSPATLSVSPGERATLSCRASTSVSHNVAWYQQKPGQAPRLLIYGASTKVTGIPARFSGSGSGTEFTLTISSLQSEDFAVYYCQHYINWPLTFGGGTKVEIKRTVAAPSVFIFPPSDEQLKSGTASVVCLLNNFYPREAKVQWKVDNALQSGNSQESVTEQDSKDSTYSLSSTLTLSKADYEKHKVYACEVTHQGLSSPVTKSFNRGEC

SEQ ID NO: 29 - protein, 453 aa, synthetic construct
QVQLQESGPGLVKPSETLSLTCTVSGYSITSDYAWNWIRQPPGKGLEWMGYISYSGSATYSPSLKSRITISRDTSKNQFSLKLSSVTAADTAVYYCARGGIAGRGRWGAMDYWGQGTTVTVSSASTKGPSVFPLAPSSKSTSGGTAALGCLVKDYFPEPVTVSWNSGALTSGVHTFPAVLQSSGLYSLSSVVTVPSSSLGTQTYICNVNHKPSNTKVDKKVEPKSCDKTHTCPPCPAPEAAGGPSVFLFPPKPKDTLMISRTPEVTCVVVDVSHEDPEVKFNWYVDGVEVHNAKTKPREEQYASTYRVVSVLTVLHQDWLNGKEYKCKVSNKALPAPIEKTISKAKGQPREPQVYTLPPSREEMTKNQVSLSCAVKGFYPSDIAVEWESNGQPENNYKTTPPVLDSDGSFFLVSKLTVDKSRWQQGNVFSCSVMHEALHNHYTQKSLSLSPGK

SEQ ID NO: 30 - protein, 214 aa, synthetic construct
DIQMTQSPSSLSASVGDRVTITCKASQNVGTNVAWYQQKPGQSPKALIYSASYRDSGVPDRFSGSGSGTDFTLTISSLQPEDFATYYCQQYKSYPLTFGQGTRLEIKRTVAAPSVFIFPPSDEQLKSGTASVVCLLNNFYPREAKVQWKVDNALQSGNSQESVTEQDSKDSTYSLSSTLTLSKADYEKHKVYACEVTHQGLSSPVTKSFNRGEC

SEQ ID NO: 31 - protein, 184 aa, Homo sapiens
MLQMAGQCSQNEYFDSLLHACIPCQLRCSSNTPPLTCQRYCNASVTNSVKGTNAILWTCLGLSLIISLAVFVLMFLLRKINSEPLKDEFKNTGSGLLGMANIDLEKSRTGDEIILPRGLEYTVEECTCEDCIKSKPKVDSDHCFPLPAMEEGATILVTTKTNDYCKSLPAALSATEIEKSISAR

SEQ ID NO: 32 - protein, 183 aa, Macaca mulatta
MLQMARQCSQNEYFDSLLHDCKPCQLRCSSTPPLTCQRYCNASMTNSVKGMNAILWTCLGLSLIISLAVFVLTFLLRKMSSEPLKDEFKNTGSGLLGMANIDLEKGRTGDEIVLPRGLEYTVEECTCEDCIKNKPKVDSDHCFPLPAMEEGATILVTTKTNDYCNSLSAALSVTEIEKSISAR

SEQ ID NO: 33 - protein, 185 aa, Mus musculus
MAQQCFHSEYFDSLLHACKPCHLRCSNPPATCQPYCDPSVTSSVKGTYTVLWIFLGLTLVLSLALFTISFLLRKMNPEALKDEPQSPGQLDGSAQLDKADTELTRIRAGDDRIFPRSLEYTVEECTCEDCVKSKPKGDSDHFFPLPAMEEGATILVTTKTGDYGKSSVPTALQSVMGMEKPTHTR

SEQ ID NO: 34 - protein, 345 aa, Homo sapiens
MYKDCIESTGDYFLLCDAEGPWGIILESLAILGIVVTILLLLAFLFLMRKIQDCSQWNVLPTQLLFLLSVLGLFGLAFAFIIELNQQTAPVRYFLFGVLFALCFSCLLAHASNLVKLVRGCVSFSWTTILCIAIGCSLLQIIIATEYVTLIMTRGMMFVNMTPCQLNVDFVVLLVYVLFLMALTFFVSKATFCGPCENWKQHGRLIFITVLFSIIIWVVWISMLLRGNPQFQRQPQWDDPVVCIALVTNAWVFLLLYIVPELCILYRSCRQECPLQGNACPVTAYQHSFQVENQELSRARDSDGAEEDVALTSYGTPIQPQTVDPTQECFIPQAKLSPQQDAGGV

SEQ ID NO: 35 - protein, 300 aa, Macaca fascicularis
MYKDCIESTGDYFLPCDSEGPWGIVLESLAILGIVVTILLLLAFLFLMRKIQDCSQWNVLPTQLLFLLSVLGLFGLAFAFIIQLNQQTAPVRYFLFGVLFALCFSCLLAHASNLVKLVRGRVSFSWTTILCIAIGCSLLQVIIAIEYVTLIMTRGMMFVHMTPYQLNVDFVVLLVYVLFLMALTFFVSKATFCGPCENWKQHGRLIFITVLFSIIIWVVWISMLLRGNPQFQRQPQWDDPVVCIALVTNAWVFLLLYIVPELCILYRSCRQECPSQGHACPVTAYQRSFQVENQELSRDC

SEQ ID NO: 36 - protein, 15 aa, synthetic construct
GGGGSGGGGSGGGGS

SEQ ID NO: 37 - protein, 20 aa, synthetic construct
GGGGSGGGGSGGGGSGGGGS